European Patent Application EP 4 772 540 A1, published July 8, 2026. Title: PROTEÍNA HÍBRIDA, SEQUÊNCIA NUCLEOTÍDICA HÍBRIDA, MOLÉCULA DE ÁCIDO NUCLEICO, VETOR PARA A EXPRESSÃO DE PROTEÍNA HÍBRIDA, USO DA PROTEÍNA HÍBRIDA OU SEQUÊNCIA NUCLEOTÍDICA, FORMULAÇÃO, PROCESSO PARA PRODUÇÃO DE UMA FORMULAÇÃO E MÉTODO PARA TRATAMENTO DE LESÕES E/OU CÂNCER CAUSADOS PELA INFECÇÃO PELO PAPILOMAVIRUS HUMANO (HPV). Applicant: UNIVERSIDADE DE SAO PAULO (USP). The sequence listing filed with the application follows.

SEQUENCE LISTING (24 sequences)

SEQ ID NO: 1 - protein, 433 aa, synthetic construct
MHHHHHHENLYFQGHGVRGKYALADASLKMADPNRFRGKDLPVLDQLTDPPGVRRVYHIQAGLPDPFQPPSLPITVYYAVLERACRSVLLNAPSEAPQIVRGASEDVRKQPYNLTIAWFRMGGNCAIPITVMEYTECSYNKSLGACPIRTQPRWNYYDSFSAVSEDNLGFLMHAPAFETAGTYLRLVKINDWTEITQFILEHRAKGSCKYALPLRIPPSACLSPQAYQQGVTVDSIGMLPRFIPENQRTVAVYSLKIAGWHGPMHGDTPTLHEYMLDLQPETTDLYCYEQLNDSSEEEDEIDGPAGQAEPDRAHYNIVTFCCKCDSTLRLCVQSTHVDIRTLEDLLMGTLGIVCPICSQKPGPKAPYTSTLLPPELSETPNATQPELAPEDPEDSALLEDPVGTVAPQIPPNWHIPSIQDAATPYHPPATPNN

SEQ ID NO: 2 - protein, 461 aa, synthetic construct
MGSSHHHHHHSSGLVPRGSHMASMTGGQQMGRGSHGVRGKYALADASLKMADPNRFRGKDLPVLDQLTDPPGVRRVYHIQAGLPDPFQPPSLPITVYYAVLERACRSVLLNAPSEAPQIVRGASEDVRKQPYNLTIAWFRMGGNCAIPITVMEYTECSYNKSLGACPIRTQPRWNYYDSFSAVSEDNLGFLMHAPAFETAGTYLRLVKINDWTEITQFILEHRAKGSCKYALPLRIPPSACLSPQAYQQGVTVDSIGMLPRFIPENQRTVAVYSLKIAGWHGPMHGDTPTLHEYMLDLQPETTDLYCYEQLNDSSEEEDEIDGPAGQAEPDRAHYNIVTFCCKCDSTLRLCVQSTHVDIRTLEDLLMGTLGIVCPICSQKPGPKAPYTSTLLPPELSETPNATQPELAPEDPEDSALLEDPVGTVAPQIPPNWHIPSIQDAATPYHPPATPNNLEHHHHHH

SEQ ID NO: 3 - protein, 443 aa, synthetic construct
MGSSHHHHHHSSGLVPRGSHMASKYALADASLKMADPNRFRGKDLPVLDQLTDPPGVRRVYHIQAGLPDPFQPPSLPITVYYAVLERACRSVLLNAPSEAPQIVRGASEDVRKQPYNLTIAWFRMGGNCAIPITVMEYTECSYNKSLGACPIRTQPRWNYYDSFSAVSEDNLGFLMHAPAFETAGTYLRLVKINDWTEITQFILEHRAKGSCKYALPLRIPPSACLSPQAYQQGVTVDSIGMLPRFIPENQRTVAVYSLKIAGWHGPLQMHGDTPTLHEYMLDLQPETTDLYGYGQLNDSSEEEDEIDGPAGQAEPDRAHYNIVTFCCKCDSTLRLCVQSTHVDIRTLEDLLMGTLGIVCPICSQKPLQGTKAPYTSTLLPPELSETPNATQPELAPEDPEDSALLEDPVGTVAPQIPPNWHIPSIQDAATPYHPPATPNNMG

SEQ ID NO: 4 - DNA, 1299 bp, synthetic construct
  source 1..1299: mol_type = other DNA
atgcaccaccaccaccaccacgaaaatctgtacttccaaggccatggggtccgcggcaaatatgccttggcggatgcctctctcaagatggccgaccccaatcgctttcgcggcaaagaccttccggtcctggaccagctgaccgaccctccgggggtccggcgcgtgtaccacatccaggcgggcctaccggacccgttccagccccccagcctcccgatcacggtttactacgccgtgttggagcgcgcctgccgcagcgtgctcctaaacgcaccgtcggaggccccccagattgtccgcggggcctccgaagacgtccggaaacaaccctacaacctgaccatcgcttggtttcggatgggaggcaactgtgctatccccatcacggtcatggagtacaccgaatgctcctacaacaagtctctgggggcctgtcccatccgaacgcagccccgctggaactactatgacagcttcagcgccgtcagcgaggataacctggggttcctgatgcacgcccccgcgtttgagaccgccggcacgtacctgcggctcgtgaagataaacgactggacggagattacacagtttatcctggagcaccgagccaagggctcctgtaagtacgccctcccgctgcgcatccccccgtcagcctgcctgtccccccaggcctaccagcagggggtgacggtggacagcatcgggatgctgccccgcttcatccccgagaaccagcgcaccgtcgccgtatacagcttgaagatcgccgggtggcacgggcccatgcatggagatacacctacattgcatgaatatatgttagatttgcaaccagagacaactgatctctactgttatgagcaattaaatgacagctcagaggaggaggatgaaatagatggtccagctggacaagcagaaccggacagagcccattacaatattgtaaccttttgttgcaagtgtgactctacgcttcggttgtgcgtacaaagcacacacgtagacattcgtactttggaagacctgttaatgggcacactaggaattgtgtgccccatctgttctcagaaaccagggcccaaggccccatacacgagcaccctgctgcccccggagctgtccgagacccccaacgccacgcagccagaactcgccccggaagaccccgaggattcggccctcttggaggaccccgtggggacggtggcgccgcaaatcccaccaaactggcacataccgtcgatccaggacgccgcgacgccttaccatcccccggccaccccgaacaac

SEQ ID NO: 5 - DNA, 1386 bp, synthetic construct
  source 1..1386: mol_type = other DNA
atgggcagcagccatcatcatcatcatcacagcagcggcctggtgccgcgcggcagccatatggctagcatgactggtggacagcaaatgggtcgcggatcccatggggtccgcggcaaatatgccttggcggatgcctctctcaagatggccgaccccaatcgctttcgcggcaaagaccttccggtcctggaccagctgaccgaccctccgggggtccggcgcgtgtaccacatccaggcgggcctaccggacccgttccagccccccagcctcccgatcacggtttactacgccgtgttggagcgcgcctgccgcagcgtgctcctaaacgcaccgtcggaggccccccagattgtccgcggggcctccgaagacgtccggaaacaaccctacaacctgaccatcgcttggtttcggatgggaggcaactgtgctatccccatcacggtcatggagtacaccgaatgctcctacaacaagtctctgggggcctgtcccatccgaacgcagccccgctggaactactatgacagcttcagcgccgtcagcgaggataacctggggttcctgatgcacgcccccgcgtttgagaccgccggcacgtacctgcggctcgtgaagataaacgactggacggagattacacagtttatcctggagcaccgagccaagggctcctgtaagtacgccctcccgctgcgcatccccccgtcagcctgcctgtccccccaggcctaccagcagggggtgacggtggacagcatcgggatgctgccccgcttcatccccgagaaccagcgcaccgtcgccgtatacagcttgaagatcgccgggtggcacgggcccatgcatggagatacacctacattgcatgaatatatgttagatttgcaaccagagacaactgatctctactgttatgagcaattaaatgacagctcagaggaggaggatgaaatagatggtccagctggacaagcagaaccggacagagcccattacaatattgtaaccttttgttgcaagtgtgactctacgcttcggttgtgcgtacaaagcacacacgtagacattcgtactttggaagacctgttaatgggcacactaggaattgtgtgccccatctgttctcagaaaccagggcccaaggccccatacacgagcaccctgctgcccccggagctgtccgagacccccaacgccacgcagccagaactcgccccggaagaccccgaggattcggccctcttggaggaccccgtggggacggtggcgccgcaaatcccaccaaactggcacataccgtcgatccaggacgccgcgacgccttaccatcccccggccaccccgaacaacctcgagcaccaccaccaccaccactga

SEQ ID NO: 6 - DNA, 1332 bp, synthetic construct
  source 1..1332: mol_type = other DNA
atgggcagcagccatcatcatcatcatcacagcagcggcctggtgccgcgcggcagccatatggctagcaagtacgcgctggcggacgcgagcctgaaaatggcggatccgaaccgtttccgtggcaaggacctgccggtgctggatcaactgaccgatccgccgggtgtgcgtcgtgtttatcacatccaagcgggtctgccggatccgtttcaaccgccgagcctgccgattaccgtgtactatgcggttctggagcgtgcgtgccgtagcgtgctgctgaacgcgccgagcgaagcgccgcagattgtgcgtggtgcgagcgaggacgttcgtaagcaaccgtacaacctgaccattgcgtggttccgtatgggtggcaactgcgcgatcccgattaccgttatggaatacaccgagtgcagctataacaaaagcctgggtgcgtgcccgatccgtacccagccgcgttggaactactatgacagcttcagcgcggtgtctgaggataacctgggtttcctgatgcatgcgccggcgtttgaaaccgcgggcacctacctgcgtctggttaagatcaacgactggaccgaaatcacccagtttattctggagcaccgtgcgaagggtagctgcaaatatgcgctgccgctgcgtattccgccgagcgcgtgcctgagcccgcaagcgtatcagcaaggtgtgaccgttgatagcatcggcatgctgccgcgttttattccggaaaaccagcgtaccgtggcggtttacagcctgaaaatcgcgggttggcatggtccgctgcagatgcatggtgacaccccgaccctgcacgaatatatgctggacctgcaaccggagaccaccgatctgtacggttatggccaactgaacgatagcagcgaggaagaggacgaaatcgatggtccggcgggtcaggcggagccggaccgtgcgcactacaacattgtgaccttctgctgcaagtgcgatagcaccctgcgtctgtgcgtgcaaagcacccacgttgacatccgtaccctggaggatctgctgatgggcaccctgggcatcgtttgcccgatttgcagccagaagccgctgcagggtaccaaagcgccgtacaccagcaccctgctgccgccggaactgagcgagaccccgaacgcgacccagccggagctggcgccggaagacccggaggatagcgcgctgctggaagatccggtgggcaccgttgcgccgcagattccgccgaactggcacatcccgagcattcaagatgcggcgaccccgtatcacccgccggcgaccccgaacaacatgggctaa

SEQ ID NO: 7 - protein, 9 aa, human papillomavirus 16
RAHYNIVTF

SEQ ID NO: 8 - protein, 34 aa, synthetic construct
MGSSHHHHHHSSGLVPRGSHMASMTGGQQMGRGS

SEQ ID NO: 9 - protein, 249 aa, Herpes simplex virus
HGVRGKYALADASLKMADPNRFRGKDLPVLDQLTDPPGVRRVYHIQAGLPDPFQPPSLPITVYYAVLERACRSVLLNAPSEAPQIVRGASEDVRKQPYNLTIAWFRMGGNCAIPITVMEYTECSYNKSLGACPIRTQPRWNYYDSFSAVSEDNLGFLMHAPAFETAGTYLRLVKINDWTEITQFILEHRAKGSCKYALPLRIPPSACLSPQAYQQGVTVDSIGMLPRFIPENQRTVAVYSLKIAGWHGP

SEQ ID NO: 10 - protein, 98 aa, human papillomavirus 16
MHGDTPTLHEYMLDLQPETTDLYCYEQLNDSSEEEDEIDGPAGQAEPDRAHYNIVTFCCKCDSTLRLCVQSTHVDIRTLEDLLMGTLGIVCPICSQKP

SEQ ID NO: 11 - protein, 72 aa, Herpes simplex virus
GPKAPYTSTLLPPELSETPNATQPELAPEDPEDSALLEDPVGTVAPQIPPNWHIPSIQDAATPYHPPATPNN

SEQ ID NO: 12 - protein, 8 aa, synthetic construct
LEHHHHHH

SEQ ID NO: 13 - protein, 23 aa, synthetic construct
MGSSHHHHHHSSGLVPRGSHMAS

SEQ ID NO: 14 - protein, 244 aa, Herpes simplex virus
KYALADASLKMADPNRFRGKDLPVLDQLTDPPGVRRVYHIQAGLPDPFQPPSLPITVYYAVLERACRSVLLNAPSEAPQIVRGASEDVRKQPYNLTIAWFRMGGNCAIPITVMEYTECSYNKSLGACPIRTQPRWNYYDSFSAVSEDNLGFLMHAPAFETAGTYLRLVKINDWTEITQFILEHRAKGSCKYALPLRIPPSACLSPQAYQQGVTVDSIGMLPRFIPENQRTVAVYSLKIAGWHGP

SEQ ID NO: 15 - protein, 98 aa, synthetic construct
MHGDTPTLHEYMLDLQPETTDLYGYGQLNDSSEEEDEIDGPAGQAEPDRAHYNIVTFCCKCDSTLRLCVQSTHVDIRTLEDLLMGTLGIVCPICSQKP

SEQ ID NO: 16 - protein, 72 aa, Herpes simplex virus
KAPYTSTLLPPELSETPNATQPELAPEDPEDSALLEDPVGTVAPQIPPNWHIPSIQDAATPYHPPATPNNMG

SEQ ID NO: 17 - RNA, 1386 nt, synthetic construct
  source 1..1386: mol_type = other RNA
atgggcagcagccatcatcatcatcatcacagcagcggcctggtgccgcgcggcagccatatggctagcatgactggtggacagcaaatgggtcgcggatcccatggggtccgcggcaaatatgccttggcggatgcctctctcaagatggccgaccccaatcgctttcgcggcaaagaccttccggtcctggaccagctgaccgaccctccgggggtccggcgcgtgtaccacatccaggcgggcctaccggacccgttccagccccccagcctcccgatcacggtttactacgccgtgttggagcgcgcctgccgcagcgtgctcctaaacgcaccgtcggaggccccccagattgtccgcggggcctccgaagacgtccggaaacaaccctacaacctgaccatcgcttggtttcggatgggaggcaactgtgctatccccatcacggtcatggagtacaccgaatgctcctacaacaagtctctgggggcctgtcccatccgaacgcagccccgctggaactactatgacagcttcagcgccgtcagcgaggataacctggggttcctgatgcacgcccccgcgtttgagaccgccggcacgtacctgcggctcgtgaagataaacgactggacggagattacacagtttatcctggagcaccgagccaagggctcctgtaagtacgccctcccgctgcgcatccccccgtcagcctgcctgtccccccaggcctaccagcagggggtgacggtggacagcatcgggatgctgccccgcttcatccccgagaaccagcgcaccgtcgccgtatacagcttgaagatcgccgggtggcacgggcccatgcatggagatacacctacattgcatgaatatatgttagatttgcaaccagagacaactgatctctactgttatgagcaattaaatgacagctcagaggaggaggatgaaatagatggtccagctggacaagcagaaccggacagagcccattacaatattgtaaccttttgttgcaagtgtgactctacgcttcggttgtgcgtacaaagcacacacgtagacattcgtactttggaagacctgttaatgggcacactaggaattgtgtgccccatctgttctcagaaaccagggcccaaggccccatacacgagcaccctgctgcccccggagctgtccgagacccccaacgccacgcagccagaactcgccccggaagaccccgaggattcggccctcttggaggaccccgtggggacggtggcgccgcaaatcccaccaaactggcacataccgtcgatccaggacgccgcgacgccttaccatcccccggccaccccgaacaacctcgagcaccaccaccaccaccactga

SEQ ID NO: 18 - RNA, 1332 nt, synthetic construct
  source 1..1332: mol_type = other RNA
atgggcagcagccatcatcatcatcatcacagcagcggcctggtgccgcgcggcagccatatggctagcaagtacgcgctggcggacgcgagcctgaaaatggcggatccgaaccgtttccgtggcaaggacctgccggtgctggatcaactgaccgatccgccgggtgtgcgtcgtgtttatcacatccaagcgggtctgccggatccgtttcaaccgccgagcctgccgattaccgtgtactatgcggttctggagcgtgcgtgccgtagcgtgctgctgaacgcgccgagcgaagcgccgcagattgtgcgtggtgcgagcgaggacgttcgtaagcaaccgtacaacctgaccattgcgtggttccgtatgggtggcaactgcgcgatcccgattaccgttatggaatacaccgagtgcagctataacaaaagcctgggtgcgtgcccgatccgtacccagccgcgttggaactactatgacagcttcagcgcggtgtctgaggataacctgggtttcctgatgcatgcgccggcgtttgaaaccgcgggcacctacctgcgtctggttaagatcaacgactggaccgaaatcacccagtttattctggagcaccgtgcgaagggtagctgcaaatatgcgctgccgctgcgtattccgccgagcgcgtgcctgagcccgcaagcgtatcagcaaggtgtgaccgttgatagcatcggcatgctgccgcgttttattccggaaaaccagcgtaccgtggcggtttacagcctgaaaatcgcgggttggcatggtccgctgcagatgcatggtgacaccccgaccctgcacgaatatatgctggacctgcaaccggagaccaccgatctgtacggttatggccaactgaacgatagcagcgaggaagaggacgaaatcgatggtccggcgggtcaggcggagccggaccgtgcgcactacaacattgtgaccttctgctgcaagtgcgatagcaccctgcgtctgtgcgtgcaaagcacccacgttgacatccgtaccctggaggatctgctgatgggcaccctgggcatcgtttgcccgatttgcagccagaagccgctgcagggtaccaaagcgccgtacaccagcaccctgctgccgccggaactgagcgagaccccgaacgcgacccagccggagctggcgccggaagacccggaggatagcgcgctgctggaagatccggtgggcaccgttgcgccgcagattccgccgaactggcacatcccgagcattcaagatgcggcgaccccgtatcacccgccggcgaccccgaacaacatgggctaa

SEQ ID NO: 19 - DNA, 1386 bp, synthetic construct
  source 1..1386: mol_type = other DNA
atgggnagyagycaycaycaycaycaycayagyagyggnctngtnccncgnggnagycayatggcnagyatgacnggnggncarcaratgggncgnggntcncayggngtncgnggnaartaygcnttrgcngaygcntcnctnaaratggcngayccnaaycgnttycgnggnaargayctnccngtnctngaycarctnacngayccnccnggngtncgncgngtntaycayathcargcnggnctnccngayccnttycarccnccnagyctnccnathacngtntaytaygcngtnttrgarcgngcntgycgnagygtnctnctnaaygcnccntcngargcnccncarathgtncgnggngcntcngargaygtncgnaarcarccntayaayctnacnathgcntggttycgnatgggnggnaaytgygcnathccnathacngtnatggartayacngartgytcntayaayaartcnctnggngcntgyccnathcgnacncarccncgntggaaytaytaygayagyttyagygcngtnagygargayaayctnggnttyctnatgcaygcnccngcnttygaracngcnggnacntayctncgnctngtnaarathaaygaytggacngarathacncarttyathctngarcaycgngcnaarggntcntgyaartaygcnctnccnctncgnathccnccntcngcntgyctntcnccncargcntaycarcarggngtnacngtngayagyathggnatgctnccncgnttyathccngaraaycarcgnacngtngcngtntayagyttraarathgcnggntggcayggnccnatgcayggngayacnccnacnttrcaygartayatgttrgayttrcarccngaracnacngayctntaytgytaygarcarttraaygayagytcngargargargaygarathgayggnccngcnggncargcngarccngayagrgcncaytayaayathgtnacnttytgytgyaartgygaytcnacnctncgnttrtgygtncaragyacncaygtngayathcgnacnttrgargayctnttratgggnacnctnggnathgtntgyccnathtgytcncaraarccnggnccnaargcnccntayacnagyacnctnctnccnccngarctntcngaracnccnaaygcnacncarccngarctngcnccngargayccngargaytcngcnctnttrgargayccngtnggnacngtngcnccncarathccnccnaaytggcayathccntcnathcargaygcngcnacnccntaycayccnccngcnacnccnaayaayctngarcaycaycaycaycaycaytga

SEQ ID NO: 20 - DNA, 1332 bp, synthetic construct
  source 1..1332: mol_type = other DNA
atgggnagyagycaycaycaycaycaycayagyagyggnctngtnccncgnggnagycayatggcnagyaartaygcnctngcngaygcnagyctnaaratggcngayccnaaycgnttycgnggnaargayctnccngtnctngaycarctnacngayccnccnggngtncgncgngtntaycayathcargcnggnctnccngayccnttycarccnccnagyctnccnathacngtntaytaygcngtnctngarcgngcntgycgnagygtnctnctnaaygcnccnagygargcnccncarathgtncgnggngcnagygargaygtncgnaarcarccntayaayctnacnathgcntggttycgnatgggnggnaaytgygcnathccnathacngtnatggartayacngartgyagytayaayaaragyctnggngcntgyccnathcgnacncarccncgntggaaytaytaygayagyttyagygcngtntcngargayaayctnggnttyctnatgcaygcnccngcnttygaracngcnggnacntayctncgnctngtnaarathaaygaytggacngarathacncarttyathctngarcaycgngcnaarggnagytgyaartaygcnctnccnctncgnathccnccnagygcntgyctnagyccncargcntaycarcarggngtnacngtngayagyathggnatgctnccncgnttyathccngaraaycarcgnacngtngcngtntayagyctnaarathgcnggntggcayggnccnctncaratgcayggngayacnccnacnctncaygartayatgctngayctncarccngaracnacngayctntayggntayggncarctnaaygayagyagygargargargaygarathgayggnccngcnggncargcngarccngaycgngcncaytayaayathgtnacnttytgytgyaartgygayagyacnctncgnctntgygtncaragyacncaygtngayathcgnacnctngargayctnctnatgggnacnctnggnathgtntgyccnathtgyagycaraarccnctncarggnacnaargcnccntayacnagyacnctnctnccnccngarctnagygaracnccnaaygcnacncarccngarctngcnccngargayccngargayagygcnctnctngargayccngtnggnacngtngcnccncarathccnccnaaytggcayathccnagyathcargaygcngcnacnccntaycayccnccngcnacnccnaayaayatgggntaa

SEQ ID NO: 21 - protein, 319 aa, Herpes simplex virus
HGVRGKYALADASLKMADPNRFRGKDLPVLDQLTDPPGVRRVYHIQAGLPDPFQPPSLPITVYYAVLERACRSVLLNAPSEAPQIVRGASEDVRKQPYNLTIAWFRMGGNCAIPITVMEYTECSYNKSLGACPIRTQPRWNYYDSFSAVSEDNLGFLMHAPAFETAGTYLRLVKINDWTEITQFILEHRAKGSCKYALPLRIPPSACLSPQAYQQGVTVDSIGMLPRFIPENQRTVAVYSLKIAGWHGPKAPYTSTLLPPELSETPNATQPELAPEDPEDSALLEDPVGTVAPQIPPNWHIPSIQDAATPYHPPATPNN

SEQ ID NO: 22 - protein, 60 aa, human papillomavirus 16
MHGDTPTLHEYMLDLQPETTDLYCYEQLNDSSEEEDEIDGPAGQAEPDRAHYNIVTFCCK

SEQ ID NO: 23 - RNA, 1386 nt, synthetic construct
  source 1..1386: mol_type = other RNA
atgggnagyagycaycaycaycaycaycayagyagyggnctngtnccncgnggnagycayatggcnagyatgacnggnggncarcaratgggncgnggntcncayggngtncgnggnaartaygcnttrgcngaygcntcnctnaaratggcngayccnaaycgnttycgnggnaargayctnccngtnctngaycarctnacngayccnccnggngtncgncgngtntaycayathcargcnggnctnccngayccnttycarccnccnagyctnccnathacngtntaytaygcngtnttrgarcgngcntgycgnagygtnctnctnaaygcnccntcngargcnccncarathgtncgnggngcntcngargaygtncgnaarcarccntayaayctnacnathgcntggttycgnatgggnggnaaytgygcnathccnathacngtnatggartayacngartgytcntayaayaartcnctnggngcntgyccnathcgnacncarccncgntggaaytaytaygayagyttyagygcngtnagygargayaayctnggnttyctnatgcaygcnccngcnttygaracngcnggnacntayctncgnctngtnaarathaaygaytggacngarathacncarttyathctngarcaycgngcnaarggntcntgyaartaygcnctnccnctncgnathccnccntcngcntgyctntcnccncargcntaycarcarggngtnacngtngayagyathggnatgctnccncgnttyathccngaraaycarcgnacngtngcngtntayagyttraarathgcnggntggcayggnccnatgcayggngayacnccnacnttrcaygartayatgttrgayttrcarccngaracnacngayctntaytgytaygarcarttraaygayagytcngargargargaygarathgayggnccngcnggncargcngarccngayagrgcncaytayaayathgtnacnttytgytgyaartgygaytcnacnctncgnttrtgygtncaragyacncaygtngayathcgnacnttrgargayctnttratgggnacnctnggnathgtntgyccnathtgytcncaraarccnggnccnaargcnccntayacnagyacnctnctnccnccngarctntcngaracnccnaaygcnacncarccngarctngcnccngargayccngargaytcngcnctnttrgargayccngtnggnacngtngcnccncarathccnccnaaytggcayathccntcnathcargaygcngcnacnccntaycayccnccngcnacnccnaayaayctngarcaycaycaycaycaycaytga

SEQ ID NO: 24 - RNA, 1332 nt, synthetic construct
  source 1..1332: mol_type = other RNA
atgggnagyagycaycaycaycaycaycayagyagyggnctngtnccncgnggnagycayatggcnagyaartaygcnctngcngaygcnagyctnaaratggcngayccnaaycgnttycgnggnaargayctnccngtnctngaycarctnacngayccnccnggngtncgncgngtntaycayathcargcnggnctnccngayccnttycarccnccnagyctnccnathacngtntaytaygcngtnctngarcgngcntgycgnagygtnctnctnaaygcnccnagygargcnccncarathgtncgnggngcnagygargaygtncgnaarcarccntayaayctnacnathgcntggttycgnatgggnggnaaytgygcnathccnathacngtnatggartayacngartgyagytayaayaaragyctnggngcntgyccnathcgnacncarccncgntggaaytaytaygayagyttyagygcngtntcngargayaayctnggnttyctnatgcaygcnccngcnttygaracngcnggnacntayctncgnctngtnaarathaaygaytggacngarathacncarttyathctngarcaycgngcnaarggnagytgyaartaygcnctnccnctncgnathccnccnagygcntgyctnagyccncargcntaycarcarggngtnacngtngayagyathggnatgctnccncgnttyathccngaraaycarcgnacngtngcngtntayagyctnaarathgcnggntggcayggnccnctncaratgcayggngayacnccnacnctncaygartayatgctngayctncarccngaracnacngayctntayggntayggncarctnaaygayagyagygargargargaygarathgayggnccngcnggncargcngarccngaycgngcncaytayaayathgtnacnttytgytgyaartgygayagyacnctncgnctntgygtncaragyacncaygtngayathcgnacnctngargayctnctnatgggnacnctnggnathgtntgyccnathtgyagycaraarccnctncarggnacnaargcnccntayacnagyacnctnctnccnccngarctnagygaracnccnaaygcnacncarccngarctngcnccngargayccngargayagygcnctnctngargayccngtnggnacngtngcnccncarathccnccnaaytggcayathccnagyathcargaygcngcnacnccntaycayccnccngcnacnccnaayaayatgggntaa